European Patent Specification EP 3 692 149 B1, published January 4, 2023. Title: Treatment of a condition associated with infection with an oncogenic bacterium. Applicant: Micreos Human Health B.V. The sequence listing filed with the application follows.

SEQUENCE LISTING (75 sequences)

SEQ ID NO: 1 - DNA, 1461 bp, Staphylococcus bacteriophage 2638A
atgctaactgctattgactatcttacgaaaaaaggttggaaaatatcatctgaccctcgcacttacgatggttaccctaaaaactacggctacagaaattaccatgaaaacggcattaattatgatgagttttgtggtggttatcatagagcttttgatgtttacagtaacgaaactaacgacgtgcctgctgttactagcggaacagttattgaagcaaacgattacggtaattttggtggtacattcgttattagagacgctaacgataacgattggatatatgggcatctacaacgtggctcaatgcgatttgttgtaggcgacaaagtcaatcaaggtgacattattggtttacaaggtaatagcaactattacgacaatcctatgagtgtacatttacatttacaattacgccctaaagacgcaaagaaagatgaaaaatcacaagtatgtagtggtttggctatggaaaaatatgacattacaaatttaaatgctaaacaagataaatcaaagaatgggagcgtgaaagagttgaaacatatctattcaaaccatattaaaggtaacaagattacagcaccaaaacctagtattcaaggtgtggtcatccacaatgattatggtagtatgacacctagtcaatacttaccatggttatatgcacgtgagaataacggtacacacgttaacggttgggctagtgtttatgcaaatagaaacgaagtgctttggtatcatccgacagactacgtagagtggcattgtggtaatcaatgggcaaatgctaacttaatcggatttgaagtgtgtgagtcgtatcctggtagaatctcggacaaattattcttagaaaatgaagaagcgacattgaaagtagctgcggatgtgatgaagtcgtacggattaccagttaatcgcaacactgtacgtctgcataacgaattcttcggaacttcttgtccacatcgttcgtgggacttgcatgttggcaaaggtgagccttacacaactactaatattaataaaatgaaagactacttcatcaaacgcatcaaacattattatgacggtggaaagctagaagtaagcaaagcagcaactatcaaacaatctgacgttaagcaagaagttaaaaagcaagaagcaaaacaaattgtgaaagcaacagattggaaacagaataaagatggcatttggtataaagctgaacatgcttcgttcacagtgacagcaccagagggaattatcacaagatacaaaggtccttggactggtcacccacaagctggtgtattacaaaaaggtcaaacgattaaatatgatgaggttcaaaaatttgacggtcatgtttgggtatcgtgggaaacgtttgagggcgaaactgtatacatgccggtacgcacatgggacgctaaaactggtaaagttggtaagttgtggggcgaaattaaataa

SEQ ID NO: 2 - protein, 486 aa, Staphylococcus bacteriophage 2638A
MLTAIDYLTKKGWKISSDPRTYDGYPKNYGYRNYHENGINYDEFCGGYHRAFDVYSNETNDVPAVTSGTVIEANDYGNFGGTFVIRDANDNDWIYGHLQRGSMRFVVGDKVNQGDIIGLQGNSNYYDNPMSVHLHLQLRPKDAKKDEKSQVCSGLAMEKYDITNLNAKQDKSKNGSVKELKHIYSNHIKGNKITAPKPSIQGVVIHNDYGSMTPSQYLPWLYARENNGTHVNGWASVYANRNEVLWYHPTDYVEWHCGNQWANANLIGFEVCESYPGRISDKLFLENEEATLKVAADVMKSYGLPVNRNTVRLHNEFFGTSCPHRSWDLHVGKGEPYTTTNINKMKDYFIKRIKHYYDGGKLEVSKAATIKQSDVKQEVKKQEAKQIVKATDWKQNKDGIWYKAEHASFTVTAPEGIITRYKGPWTGHPQAGVLQKGQTIKYDEVQKFDGHVWVSWETFEGETVYMPVRTWDAKTGKVGKLWGEIK

SEQ ID NO: 3 - DNA, 279 bp, Staphylococcus simulans
tggaaaacaaacaaatatggcacactatataaatcagagtcagctagcttcacacctaatacagatataataacaagaacgactggtccatttagaagcatgccgcagtcaggagtcttaaaagcaggtcaaacaattcattatgatgaagtgatgaaacaagacggtcatgtttgggtaggttatacaggtaacagtggccaacgtatttacttgcctgtaagaacatggaataaatctactaatactttaggtgttctttggggaactataaagtga

SEQ ID NO: 4 - protein, 92 aa, Staphylococcus simulans
WKTNKYGTLYKSESASFTPNTDIITRTTGPFRSMPQSGVLKAGQTIHYDEVMKQDGHVWVGYTGNSGQRIYLPVRTWNKSTNTLGVLWGTIK

SEQ ID NO: 5 - DNA, 285 bp, Staphylococcus bacteriophage 2638A
tggaaacagaataaagatggcatttggtataaagctgaacatgcttcgttcacagtgacagcaccagagggaattatcacaagatacaaaggtccttggactggtcacccacaagctggtgtattacaaaaaggtcaaacgattaaatatgatgaggttcaaaaatttgacggtcatgtttgggtatcgtgggaaacgtttgagggcgaaactgtatacatgccggtacgcacatgggacgctaaaactggtaaagttggtaagttgtggggcgaaattaaataa

SEQ ID NO: 6 - protein, 94 aa, Staphylococcus bacteriophage 2638A
WKQNKDGIWYKAEHASFTVTAPEGIITRYKGPWTGHPQAGVLQKGQTIKYDEVQKFDGHVWVSWETFEGETVYMPVRTWDAKTGKVGKLWGEIK

SEQ ID NO: 7 - DNA, 282 bp, Staphylococcus bacteriophage phiNM3
ggtaaatctgcaagtaaaataacagttggaagtaaagcgccttataaccttaaatggtcaaaaggtgcttattttaatgcgaaaatcgacggcttaggtgctacttcagccactagatacggtgataatcgtactaactatagattcgatgttggacaggctgtatacgcgcctggaacattaatatatgtgtttgaaattatagatggttggtgtcgcatttattggaacaatcataatgagtggatatggcatgagagattgattgtgaaagaagtgttt

SEQ ID NO: 8 - protein, 94 aa, Staphylococcus bacteriophage phiNM3
GKSASKITVGSKAPYNLKWSKGAYFNAKIDGLGATSATRYGDNRTNYRFDVGQAVYAPGTLIYVFEIIDGWCRIYWNNHNEWIWHERLIVKEVF

SEQ ID NO: 9 - DNA, 585 bp, Staphylococcus bacteriophage K
atggctaagactcaagcagaaataaataaacgtttagatgcttatgcaaaaggaacagtagatagcccttacagagttaaaaaagctacaagttatgacccatcatttggtgtaatggaagcaggagccattgatgcagatggttactatcacgctcagtgtcaagaccttattacagactatgttttatggttaacagataataaagttagaacttggggtaatgctaaagaccaaattaaacagagttatggtactggatttaaaatacatgaaaataaaccttctactgtacctaaaaaaggttggattgcggtatttacatccggtagttatgaacagtggggtcacataggtattgtatatgatggaggtaatacttctacatttactattttagagcaaaactggaatggttatgctaataaaaaacctacaaaacgtgtagataattattacggattaactcacttcattgaaatacctgtaaaagcaggaactactgttaaaaaagaaacagctaagaaaagcgcaagtaaaacgcctgcacctaaaaagaaagcaacactaaaagtttctaagaat

SEQ ID NO: 10 - protein, 195 aa, Staphylococcus bacteriophage K
MAKTQAEINKRLDAYAKGTVDSPYRVKKATSYDPSFGVMEAGAIDADGYYHAQCQDLITDYVLWLTDNKVRTWGNAKDQIKQSYGTGFKIHENKPSTVPKKGWIAVFTSGSYEQWGHIGIVYDGGNTSTFTILEQNWNGYANKKPTKRVDNYYGLTHFIEIPVKAGTTVKKETAKKSASKTPAPKKKATLKVSKN

SEQ ID NO: 11 - DNA, 420 bp, Staphylococcus bacteriophage Twort
atgaaaaccctgaaacaagcagagtcctacattaagagtaaagtaaatacaggaactgattttgatggtttatatgggtatcagtgtatggacttagcagtagattatatttaccatgtaacagatggtaaaataagaatgtggggtaatgctaaggatgcgataaataactcttttggtggtactgctacggtatataaaaactaccctgcttttagacctaagtacggtgatgtagtcgtatggactactggtaattttgcaacttatggtcatatcgcaatagttactaaccctgacccttatggagaccttcaatatgttacagttcttgaacaaaactggaacggtaacgggatttataaaaccgagttagctacaatcagaacacacgattacacaggaattacacattttatt

SEQ ID NO: 12 - protein, 140 aa, Staphylococcus bacteriophage Twort
MKTLKQAESYIKSKVNTGTDFDGLYGYQCMDLAVDYIYHVTDGKIRMWGNAKDAINNSFGGTATVYKNYPAFRPKYGDVVVWTTGNFATYGHIAIVTNPDPYGDLQYVTVLEQNWNGNGIYKTELATIRTHDYTGITHFI

SEQ ID NO: 13 - DNA, 438 bp, Staphylococcus bacteriophage 2638A
atgctaactgctattgactatcttacgaaaaaaggttggaaaatatcatctgaccctcgcacttacgatggttaccctaaaaactacggctacagaaattaccatgaaaacggcattaattatgatgagttttgtggtggttatcatagagcttttgatgtttacagtaacgaaactaacgacgtgcctgctgttactagcggaacagttattgaagcaaacgattacggtaattttggtggtacattcgttattagagacgctaacgataacgattggatatatgggcatctacaacgtggctcaatgcgatttgttgtaggcgacaaagtcaatcaaggtgacattattggtttacaaggtaatagcaactattacgacaatcctatgagtgtacatttacatttacaattacgccctaaagacgcaaagaaagat

SEQ ID NO: 14 - protein, 146 aa, Staphylococcus bacteriophage 2638A
MLTAIDYLTKKGWKISSDPRTYDGYPKNYGYRNYHENGINYDEFCGGYHRAFDVYSNETNDVPAVTSGTVIEANDYGNFGGTFVIRDANDNDWIYGHLQRGSMRFVVGDKVNQGDIIGLQGNSNYYDNPMSVHLHLQLRPKDAKKD

SEQ ID NO: 15 - DNA, 420 bp, Staphylococcus simulans
gctgcaacacatgaacattcagcacaatggttgaataattacaaaaaaggatatggttacggtccttatccattaggtataaatggcggtatgcactacggagttgatttttttatgaatattggaacaccagtaaaagctatttcaagcggaaaaatagttgaagctggttggagtaattacggaggaggtaatcaaataggtcttattgaaaatgatggagtgcatagacaatggtatatgcatctaagtaaatataatgttaaagtaggagattatgtcaaagctggtcaaataatcggttggtctggaagcactggttattctacagcaccacatttacacttccaaagaatggttaattcattttcaaattcaactgcccaagatccaatgcctttcttaaagagcgcaggatat

SEQ ID NO: 16 - protein, 140 aa, Staphylococcus simulans
AATHEHSAQWLNNYKKGYGYGPYPLGINGGMHYGVDFFMNIGTPVKAISSGKIVEAGWSNYGGGNQIGLIENDGVHRQWYMHLSKYNVKVGDYVKAGQIIGWSGSTGYSTAPHLHFQRMVNSFSNSTAQDPMPFLKSAGY

SEQ ID NO: 17 - DNA, 510 bp, Staphylococcus bacteriophage 2638A
ggtaacaagattacagcaccaaaacctagtattcaaggtgtggtcatccacaatgattatggtagtatgacacctagtcaatacttaccatggttatatgcacgtgagaataacggtacacacgttaacggttgggctagtgtttatgcaaatagaaacgaagtgctttggtatcatccgacagactacgtagagtggcattgtggtaatcaatgggcaaatgctaacttaatcggatttgaagtgtgtgagtcgtatcctggtagaatctcggacaaattattcttagaaaatgaagaagcgacattgaaagtagctgcggatgtgatgaagtcgtacggattaccagttaatcgcaacactgtacgtctgcataacgaattcttcggaacttcttgtccacatcgttcgtgggacttgcatgttggcaaaggtgagccttacacaactactaatattaataaaatgaaagactacttcatcaaacgcatcaaacattattatgacggt

SEQ ID NO: 18 - protein, 169 aa, Staphylococcus bacteriophage 2638A
NKITAPKPSIQGVVIHNDYGSMTPSQYLPWLYARENNGTHVNGWASVYANRNEVLWYHPTDYVEWHCGNQWANANLIGFEVCESYPGRISDKLFLENEEATLKVAADVMKSYGLPVNRNTVRLHNEFFGTSCPHRSWDLHVGKGEPYTTTNINKMKDYFIKRIKHYYDG

SEQ ID NO: 19 - DNA, 1407 bp, Artificial Sequence
  artificial construct
atggctaagactcaagcagaaataaataaacgtttagatgcttatgcaaaaggaacagtagatagcccttacagagttaaaaaagctacaagttatgacccatcatttggtgtaatggaagcaggagccattgatgcagatggttactatcacgctcagtgtcaagaccttattacagactatgttttatggttaacagataataaagttagaacttggggtaatgctaaagaccaaattaaacagagttatggtactggatttaaaatacatgaaaataaaccttctactgtacctaaaaaaggttggattgcggtatttacatccggtagttatgaacagtggggtcacataggtattgtatatgatggaggtaatacttctacatttactattttagagcaaaactggaatggttatgctaataaaaaacctacaaaacgtgtagataattattacggattaactcacttcattgaaatacctgtaaaagcaggaactactgttaaaaaagaaacagctaagaaaagcgcaagtaaaacgcctgcacctaaaaagaaagcaacactaaaagtttctaagaatgagctcatggctaagactcaagcagaaataaataaacgtttagatgcttatgcaaaaggaacagtagatagcccttacagagttaaaaaagctacaagttatgacccatcatttggtgtaatggaagcaggagccattgatgcagatggttactatcacgctcagtgtcaagaccttattacagactatgttttatggttaacagataataaagttagaacttggggtaatgctaaagaccaaattaaacagagttatggtactggatttaaaatacatgaaaataaaccttctactgtacctaaaaaaggttggattgcggtatttacatccggtagttatgaacagtggggtcacataggtattgtatatgatggaggtaatacttctacatttactattttagagcaaaactggaatggttatgctaataaaaaacctacaaaacgtgtagataattattacggattaactcacttcattgaaatacctgtaaaagcaggaaaagcaggtggtacagtaactccaacgccgaatacaggttggaaaacaaacaaatatggcacactatataaatcagagtcagctagcttcacacctaatacagatataataacaagaacgactggtccatttagaagcatgccgcagtcaggagtcttaaaagcaggtcaaacaattcattatgatgaagtgatgaaacaagacggtcatgtttgggtaggttatacaggtaacagtggccaacgtatttacttgcctgtaagaacatggaataaatctactaatactttaggtgttctttggggaactataaagtaa

SEQ ID NO: 20 - protein, 468 aa, Artificial Sequence
  artificial construct
MAKTQAEINKRLDAYAKGTVDSPYRVKKATSYDPSFGVMEAGAIDADGYYHAQCQDLITDYVLWLTDNKVRTWGNAKDQIKQSYGTGFKIHENKPSTVPKKGWIAVFTSGSYEQWGHIGIVYDGGNTSTFTILEQNWNGYANKKPTKRVDNYYGLTHFIEIPVKAGTTVKKETAKKSASKTPAPKKKATLKVSKNELMAKTQAEINKRLDAYAKGTVDSPYRVKKATSYDPSFGVMEAGAIDADGYYHAQCQDLITDYVLWLTDNKVRTWGNAKDQIKQSYGTGFKIHENKPSTVPKKGWIAVFTSGSYEQWGHIGIVYDGGNTSTFTILEQNWNGYANKKPTKRVDNYYGLTHFIEIPVKAGKAGGTVTPTPNTGWKTNKYGTLYKSESASFTPNTDIITRTTGPFRSMPQSGVLKAGQTIHYDEVMKQDGHVWVGYTGNSGQRIYLPVRTWNKSTNTLGVLWGTIK

SEQ ID NO: 21 - DNA, 1209 bp, Artificial Sequence
  artificial construct
gctgcaacacatgaacattcagcacaatggttgaataattacaaaaaaggatatggttacggtccttatccattaggtataaatggcggtatgcactacggagttgatttttttatgaatattggaacaccagtaaaagctatttcaagcggaaaaatagttgaagctggttggagtaattacggaggaggtaatcaaataggtcttattgaaaatgatggagtgcatagacaatggtatatgcatctaagtaaatataatgttaaagtaggagattatgtcaaagctggtcaaataatcggttggtctggaagcactggttattctacagcaccacatttacacttccaaagaatggttaattcattttcaaattcaactgcccaagatccaatgcctttcttaaagagcgcaggatatggaaaagcaggtggtacagtaactccaacgccgaatacaggtgagctcgctgcaacacatgaacattcagcacaatggttgaataattacaaaaaaggatatggttacggtccttatccattaggtataaatggcggtatgcactacggagttgatttttttatgaatattggaacaccagtaaaagctatttcaagcggaaaaatagttgaagctggttggagtaattacggaggaggtaatcaaataggtcttattgaaaatgatggagtgcatagacaatggtatatgcatctaagtaaatataatgttaaagtaggagattatgtcaaagctggtcaaataatcggttggtctggaagcactggttattctacagcaccacatttacacttccaaagaatggttaattcattttcaaattcaactgcccaagatccaatgcctttcttaaagagcgcaggatatggaaaagcaggtggtacagtaactccaacgccgaatacaggttggaaaacaaacaaatatggcacactatataaatcagagtcagctagcttcacacctaatacagatataataacaagaacgactggtccatttagaagcatgccgcagtcaggagtcttaaaagcaggtcaaacaattcattatgatgaagtgatgaaacaagacggtcatgtttgggtaggttatacaggtaacagtggccaacgtatttacttgcctgtaagaacatggaataaatctactaatactttaggtgttctttggggaactataaagtaa

SEQ ID NO: 22 - protein, 402 aa, Artificial Sequence
  artificial construct
AATHEHSAQWLNNYKKGYGYGPYPLGINGGMHYGVDFFMNIGTPVKAISSGKIVEAGWSNYGGGNQIGLIENDGVHRQWYMHLSKYNVKVGDYVKAGQIIGWSGSTGYSTAPHLHFQRMVNSFSNSTAQDPMPFLKSAGYGKAGGTVTPTPNTGELAATHEHSAQWLNNYKKGYGYGPYPLGINGGMHYGVDFFMNIGTPVKAISSGKIVEAGWSNYGGGNQIGLIENDGVHRQWYMHLSKYNVKVGDYVKAGQIIGWSGSTGYSTAPHLHFQRMVNSFSNSTAQDPMPFLKSAGYGKAGGTVTPTPNTGWKTNKYGTLYKSESASFTPNTDIITRTTGPFRSMPQSGVLKAGQTIHYDEVMKQDGHVWVGYTGNSGQRIYLPVRTWNKSTNTLGVLWGTIK

SEQ ID NO: 23 - DNA, 1686 bp, Artificial Sequence
  artificial construct
gcaaagaaagatgaaaaatcacaagtatgtagtggtttggctatggaaaaatatgacattacaaatttaaatgctaaacaagataaatcaaagaatgggagcgtgaaagagttgaaacatatctattcaaaccatattaaaggtaacaagattacagcaccaaaacctagtattcaaggtgtggtcatccacaatgattatggtagtatgacacctagtcaatacttaccatggttatatgcacgtgagaataacggtacacacgttaacggttgggctagtgtttatgcaaatagaaacgaagtgctttggtatcatccgacagactacgtagagtggcattgtggtaatcaatgggcaaatgctaacttaatcggatttgaagtgtgtgagtcgtatcctggtagaatctcggacaaattattcttagaaaatgaagaagcgacattgaaagtagctgcggatgtgatgaagtcgtacggattaccagttaatcgcaacactgtacgtctgcataacgaattcttcggaacttcttgtccacatcgttcgtgggacttgcatgttggcaaaggtgagccttacacaactactaatattaataaaatgaaagactacttcatcaaacgcatcaaacattattatgacggtgagctcgcaaagaaagatgaaaaatcacaagtatgtagtggtttggctatggaaaaatatgacattacaaatttaaatgctaaacaagataaatcaaagaatgggagcgtgaaagagttgaaacatatctattcaaaccatattaaaggtaacaagattacagcaccaaaacctagtattcaaggtgtggtcatccacaatgattatggtagtatgacacctagtcaatacttaccatggttatatgcacgtgagaataacggtacacacgttaacggttgggctagtgtttatgcaaatagaaacgaagtgctttggtatcatccgacagactacgtagagtggcattgtggtaatcaatgggcaaatgctaacttaatcggatttgaagtgtgtgagtcgtatcctggtagaatctcggacaaattattcttagaaaatgaagaagcgacattgaaagtagctgcggatgtgatgaagtcgtacggattaccagttaatcgcaacactgtacgtctgcataacgaattcttcggaacttcttgtccacatcgttcgtgggacttgcatgttggcaaaggtgagccttacacaactactaatattaataaaatgaaagactacttcatcaaacgcatcaaacattattatgacggtggaaagctagaagtaagcaaagcagcaactatcaaacaatctgacgttaagcaagaagttaaaaagcaagaagcaaaacaaattgtgaaagcaacagattggaaaacaaacaaatatggcacactatataaatcagagtcagctagcttcacacctaatacagatataataacaagaacgactggtccatttagaagcatgccgcagtcaggagtcttaaaagcaggtcaaacaattcattatgatgaagtgatgaaacaagacggtcatgtttgggtaggttatacaggtaacagtggccaacgtatttacttgcctgtaagaacatggaataaatctactaatactttaggtgttctttggggaactataaagtaa

SEQ ID NO: 24 - protein, 561 aa, Artificial Sequence
  artificial construct
AKKDEKSQVCSGLAMEKYDITNLNAKQDKSKNGSVKELKHIYSNHIKGNKITAPKPSIQGVVIHNDYGSMTPSQYLPWLYARENNGTHVNGWASVYANRNEVLWYHPTDYVEWHCGNQWANANLIGFEVCESYPGRISDKLFLENEEATLKVAADVMKSYGLPVNRNTVRLHNEFFGTSCPHRSWDLHVGKGEPYTTTNINKMKDYFIKRIKHYYDGELAKKDEKSQVCSGLAMEKYDITNLNAKQDKSKNGSVKELKHIYSNHIKGNKITAPKPSIQGVVIHNDYGSMTPSQYLPWLYARENNGTHVNGWASVYANRNEVLWYHPTDYVEWHCGNQWANANLIGFEVCESYPGRISDKLFLENEEATLKVAADVMKSYGLPVNRNTVRLHNEFFGTSCPHRSWDLHVGKGEPYTTTNINKMKDYFIKRIKHYYDGGKLEVSKAATIKQSDVKQEVKKQEAKQIVKATDWKTNKYGTLYKSESASFTPNTDIITRTTGPFRSMPQSGVLKAGQTIHYDEVMKQDGHVWVGYTGNSGQRIYLPVRTWNKSTNTLGVLWGTIK

SEQ ID NO: 25 - DNA, 1131 bp, Artificial Sequence
  artificial construct
atgagaggatcgcatcaccatcaccatcacggatctggctctggatctggtatcgagggaaggccttataatggaactggatccgcatgcgagctcgcaaagaaagatgaaaaatcacaagtatgtagtggtttggctatggaaaaatatgacattacaaatttaaatgctaaacaagataaatcaaagaatgggagcgtgaaagagttgaaacatatctattcaaaccatattaaaggtaacaagattacagcaccaaaacctagtattcaaggtgtggtcatccacaatgattatggtagtatgacacctagtcaatacttaccatggttatatgcacgtgagaataacggtacacacgttaacggttgggctagtgtttatgcaaatagaaacgaagtgctttggtatcatccgacagactacgtagagtggcattgtggtaatcaatgggcaaatgctaacttaatcggatttgaagtgtgtgagtcgtatcctggtagaatctcggacaaattattcttagaaaatgaagaagcgacattgaaagtagctgcggatgtgatgaagtcgtacggattaccagttaatcgcaacactgtacgtctgcataacgaattcttcggaacttcttgtccacatcgttcgtgggacttgcatgttggcaaaggtgagccttacacaactactaatattaataaaatgaaagactacttcatcaaacgcatcaaacattattatgacggtggaaagctagaagtaagcaaagcagcaactatcaaacaatctgacgttaagcaagaagttaaaaagcaagaagcaaaacaaattgtgaaagcaacagattggaaacagaataaagatggcatttggtataaagctgaacatgcttcgttcacagtgacagcaccagagggaattatcacaagatacaaaggtccttggactggtcacccacaagctggtgtattacaaaaaggtcaaacgattaaatatgatgaggttcaaaaatttgacggtcatgtttgggtatcgtgggaaacgtttgagggcgaaactgtatacatgccggtacgcacatgggacgctaaaactggtaaagttggtaagttgtggggcgaaattaaataa

SEQ ID NO: 26 - protein, 376 aa, Artificial Sequence
  artificial construct
MRGSHHHHHHGSGSGSGIEGRPYNGTGSACELAKKDEKSQVCSGLAMEKYDITNLNAKQDKSKNGSVKELKHIYSNHIKGNKITAPKPSIQGVVIHNDYGSMTPSQYLPWLYARENNGTHVNGWASVYANRNEVLWYHPTDYVEWHCGNQWANANLIGFEVCESYPGRISDKLFLENEEATLKVAADVMKSYGLPVNRNTVRLHNEFFGTSCPHRSWDLHVGKGEPYTTTNINKMKDYFIKRIKHYYDGGKLEVSKAATIKQSDVKQEVKKQEAKQIVKATDWKQNKDGIWYKAEHASFTVTAPEGIITRYKGPWTGHPQAGVLQKGQTIKYDEVQKFDGHVWVSWETFEGETVYMPVRTWDAKTGKVGKLWGEIK

SEQ ID NO: 27 - DNA, 1125 bp, Artificial Sequence
  artificial construct
atgagaggatcgcatcaccatcaccatcacggatctggctctggatctggtatcgagggaaggccttataatggaactggatccgcatgcgagctcgcaaagaaagatgaaaaatcacaagtatgtagtggtttggctatggaaaaatatgacattacaaatttaaatgctaaacaagataaatcaaagaatgggagcgtgaaagagttgaaacatatctattcaaaccatattaaaggtaacaagattacagcaccaaaacctagtattcaaggtgtggtcatccacaatgattatggtagtatgacacctagtcaatacttaccatggttatatgcacgtgagaataacggtacacacgttaacggttgggctagtgtttatgcaaatagaaacgaagtgctttggtatcatccgacagactacgtagagtggcattgtggtaatcaatgggcaaatgctaacttaatcggatttgaagtgtgtgagtcgtatcctggtagaatctcggacaaattattcttagaaaatgaagaagcgacattgaaagtagctgcggatgtgatgaagtcgtacggattaccagttaatcgcaacactgtacgtctgcataacgaattcttcggaacttcttgtccacatcgttcgtgggacttgcatgttggcaaaggtgagccttacacaactactaatattaataaaatgaaagactacttcatcaaacgcatcaaacattattatgacggtggaaagctagaagtaagcaaagcagcaactatcaaacaatctgacgttaagcaagaagttaaaaagcaagaagcaaaacaaattgtgaaagcaacagattggaaaacaaacaaatatggcacactatataaatcagagtcagctagcttcacacctaatacagatataataacaagaacgactggtccatttagaagcatgccgcagtcaggagtcttaaaagcaggtcaaacaattcattatgatgaagtgatgaaacaagacggtcatgtttgggtaggttatacaggtaacagtggccaacgtatttacttgcctgtaagaacatggaataaatctactaatactttaggtgttctttggggaactataaagtaa

SEQ ID NO: 28 - protein, 374 aa, Artificial Sequence
  artificial construct
MRGSHHHHHHGSGSGSGIEGRPYNGTGSACELAKKDEKSQVCSGLAMEKYDITNLNAKQDKSKNGSVKELKHIYSNHIKGNKITAPKPSIQGVVIHNDYGSMTPSQYLPWLYARENNGTHVNGWASVYANRNEVLWYHPTDYVEWHCGNQWANANLIGFEVCESYPGRISDKLFLENEEATLKVAADVMKSYGLPVNRNTVRLHNEFFGTSCPHRSWDLHVGKGEPYTTTNINKMKDYFIKRIKHYYDGGKLEVSKAATIKQSDVKQEVKKQEAKQIVKATDWKTNKYGTLYKSESASFTPNTDIITRTTGPFRSMPQSGVLKAGQTIHYDEVMKQDGHVWVGYTGNSGQRIYLPVRTWNKSTNTLGVLWGTIK

SEQ ID NO: 29 - DNA, 1131 bp, Artificial Sequence
  artificial construct
atgagaggatcgcatcaccatcaccatcacggatctggctctggatctggtatcgagggaaggccttataatggaactggatccgcatgcgagctcgcaaagaaagatgaaaaatcacaagtatgtagtggtttggctatggaaaaatatgacattacaaatttaaatgctaaacaagataaatcaaagaatgggagcgtgaaagagttgaaacatatctattcaaaccatattaaaggtaacaagattacagcaccaaaacctagtattcaaggtgtggtcatccacaatgattatggtagtatgacacctagtcaatacttaccatggttatatgcacgtgagaataacggtacacacgttaacggttgggctagtgtttatgcaaatagaaacgaagtgctttggtatcatccgacagactacgtagagtggcattgtggtaatcaatgggcaaatgctaacttaatcggatttgaagtgtgtgagtcgtatcctggtagaatctcggacaaattattcttagaaaatgaagaagcgacattgaaagtagctgcggatgtgatgaagtcgtacggattaccagttaatcgcaacactgtacgtctgcataacgaattcttcggaacttcttgtccacatcgttcgtgggacttgcatgttggcaaaggtgagccttacacaactactaatattaataaaatgaaagactacttcatcaaacgcatcaaacattattatgacggtggaaagctagaagtaagcaaagcagcaactatcaaacaatctgacgttaagcaagaagttaaaaagcaagaagcaaaacaaattgtgaaagcaacagatggtaaatctgcaagtaaaataacagttggaagtaaagcgccttataaccttaaatggtcaaaaggtgcttattttaatgcgaaaatcgacggcttaggtgctacttcagccactagatacggtgataatcgtactaactatagattcgatgttggacaggctgtatacgcgcctggaacattaatatatgtgtttgaaattatagatggttggtgtcgcatttattggaacaatcataatgagtggatatggcatgagagattgattgtgaaagaagtgttttaa

SEQ ID NO: 30 - protein, 376 aa, Artificial Sequence
  artificial construct
MRGSHHHHHHGSGSGSGIEGRPYNGTGSACELAKKDEKSQVCSGLAMEKYDITNLNAKQDKSKNGSVKELKHIYSNHIKGNKITAPKPSIQGVVIHNDYGSMTPSQYLPWLYARENNGTHVNGWASVYANRNEVLWYHPTDYVEWHCGNQWANANLIGFEVCESYPGRISDKLFLENEEATLKVAADVMKSYGLPVNRNTVRLHNEFFGTSCPHRSWDLHVGKGEPYTTTNINKMKDYFIKRIKHYYDGGKLEVSKAATIKQSDVKQEVKKQEAKQIVKATDGKSASKITVGSKAPYNLKWSKGAYFNAKIDGLGATSATRYGDNRTNYRFDVGQAVYAPGTLIYVFEIIDGWCRIYWNNHNEWIWHERLIVKEVF

SEQ ID NO: 31 - DNA, 975 bp, Artificial Sequence
  artificial construct
atgagaggatcgcatcaccatcaccatcacggatctggctctggatctggtatcgagggaaggccttataatggaactggatccgcatgcgagctcatggctaagactcaagcagaaataaataaacgtttagatgcttatgcaaaaggaacagtagatagcccttacagagttaaaaaagctacaagttatgacccatcatttggtgtaatggaagcaggagccattgatgcagatggttactatcacgctcagtgtcaagaccttattacagactatgttttatggttaacagataataaagttagaacttggggtaatgctaaagaccaaattaaacagagttatggtactggatttaaaatacatgaaaataaaccttctactgtacctaaaaaaggttggattgcggtatttacatccggtagttatgaacagtggggtcacataggtattgtatatgatggaggtaatacttctacatttactattttagagcaaaactggaatggttatgctaataaaaaacctacaaaacgtgtagataattattacggattaactcacttcattgaaatacctgtaaaagcaggaaagctagaagtaagcaaagcagcaactatcaaacaatctgacgttaagcaagaagttaaaaagcaagaagcaaaacaaattgtgaaagcaacagattggaaacagaataaagatggcatttggtataaagctgaacatgcttcgttcacagtgacagcaccagagggaattatcacaagatacaaaggtccttggactggtcacccacaagctggtgtattacaaaaaggtcaaacgattaaatatgatgaggttcaaaaatttgacggtcatgtttgggtatcgtgggaaacgtttgagggcgaaactgtatacatgccggtacgcacatgggacgctaaaactggtaaagttggtaagttgtggggcgaaattaaataa

SEQ ID NO: 32 - protein, 324 aa, Artificial Sequence
  artificial construct
MRGSHHHHHHGSGSGSGIEGRPYNGTGSACELMAKTQAEINKRLDAYAKGTVDSPYRVKKATSYDPSFGVMEAGAIDADGYYHAQCQDLITDYVLWLTDNKVRTWGNAKDQIKQSYGTGFKIHENKPSTVPKKGWIAVFTSGSYEQWGHIGIVYDGGNTSTFTILEQNWNGYANKKPTKRVDNYYGLTHFIEIPVKAGKLEVSKAATIKQSDVKQEVKKQEAKQIVKATDWKQNKDGIWYKAEHASFTVTAPEGIITRYKGPWTGHPQAGVLQKGQTIKYDEVQKFDGHVWVSWETFEGETVYMPVRTWDAKTGKVGKLWGEIK

SEQ ID NO: 33 - DNA, 912 bp, Artificial Sequence
  artificial construct
atgagaggatcgcatcaccatcaccatcacggatctggctctggatctggtatcgagggaaggccttataatggaactggatccgcatgcgagctcatggctaagactcaagcagaaataaataaacgtttagatgcttatgcaaaaggaacagtagatagcccttacagagttaaaaaagctacaagttatgacccatcatttggtgtaatggaagcaggagccattgatgcagatggttactatcacgctcagtgtcaagaccttattacagactatgttttatggttaacagataataaagttagaacttggggtaatgctaaagaccaaattaaacagagttatggtactggatttaaaatacatgaaaataaaccttctactgtacctaaaaaaggttggattgcggtatttacatccggtagttatgaacagtggggtcacataggtattgtatatgatggaggtaatacttctacatttactattttagagcaaaactggaatggttatgctaataaaaaacctacaaaacgtgtagataattattacggattaactcacttcattgaaatacctgtaaaagcaggaaaagcaggtggtacagtaactccaacgccgaatacaggttggaaaacaaacaaatatggcacactatataaatcagagtcagctagcttcacacctaatacagatataataacaagaacgactggtccatttagaagcatgccgcagtcaggagtcttaaaagcaggtcaaacaattcattatgatgaagtgatgaaacaagacggtcatgtttgggtaggttatacaggtaacagtggccaacgtatttacttgcctgtaagaacatggaataaatctactaatactttaggtgttctttggggaactataaagtaa

SEQ ID NO: 34 - protein, 303 aa, Artificial Sequence
  artificial construct
MRGSHHHHHHGSGSGSGIEGRPYNGTGSACELMAKTQAEINKRLDAYAKGTVDSPYRVKKATSYDPSFGVMEAGAIDADGYYHAQCQDLITDYVLWLTDNKVRTWGNAKDQIKQSYGTGFKIHENKPSTVPKKGWIAVFTSGSYEQWGHIGIVYDGGNTSTFTILEQNWNGYANKKPTKRVDNYYGLTHFIEIPVKAGKAGGTVTPTPNTGWKTNKYGTLYKSESASFTPNTDIITRTTGPFRSMPQSGVLKAGQTIHYDEVMKQDGHVWVGYTGNSGQRIYLPVRTWNKSTNTLGVLWGTIK

SEQ ID NO: 35 - DNA, 966 bp, Artificial Sequence
  artificial construct
atgagaggatcgcatcaccatcaccatcacggatctggctctggatctggtatcgagggaaggccttataatggaactggatccgcatgcgagctcatggctaagactcaagcagaaataaataaacgtttagatgcttatgcaaaaggaacagtagatagcccttacagagttaaaaaagctacaagttatgacccatcatttggtgtaatggaagcaggagccattgatgcagatggttactatcacgctcagtgtcaagaccttattacagactatgttttatggttaacagataataaagttagaacttggggtaatgctaaagaccaaattaaacagagttatggtactggatttaaaatacatgaaaataaaccttctactgtacctaaaaaaggttggattgcggtatttacatccggtagttatgaacagtggggtcacataggtattgtatatgatggaggtaatacttctacatttactattttagagcaaaactggaatggttatgctaataaaaaacctacaaaacgtgtagataattattacggattaactcacttcattgaaatacctgtaaaagcaggaactactgttaaaaaagaaacagctaagaaaagcgcaagtaaaacgcctgcacctaaaaagaaagcaacactaaaagtttctaagaatggtaaatctgcaagtaaaataacagttggaagtaaagcgccttataaccttaaatggtcaaaaggtgcttattttaatgcgaaaatcgacggcttaggtgctacttcagccactagatacggtgataatcgtactaactatagattcgatgttggacaggctgtatacgcgcctggaacattaatatatgtgtttgaaattatagatggttggtgtcgcatttattggaacaatcataatgagtggatatggcatgagagattgattgtgaaagaagtgttttaa

SEQ ID NO: 36 - protein, 321 aa, Artificial Sequence
  artificial construct
MRGSHHHHHHGSGSGSGIEGRPYNGTGSACELMAKTQAEINKRLDAYAKGTVDSPYRVKKATSYDPSFGVMEAGAIDADGYYHAQCQDLITDYVLWLTDNKVRTWGNAKDQIKQSYGTGFKIHENKPSTVPKKGWIAVFTSGSYEQWGHIGIVYDGGNTSTFTILEQNWNGYANKKPTKRVDNYYGLTHFIEIPVKAGTTVKKETAKKSASKTPAPKKKATLKVSKNGKSASKITVGSKAPYNLKWSKGAYFNAKIDGLGATSATRYGDNRTNYRFDVGQAVYAPGTLIYVFEIIDGWCRIYWNNHNEWIWHERLIVKEVF

SEQ ID NO: 37 - DNA, 927 bp, Artificial Sequence
  artificial construct
atgagaggatcgcatcaccatcaccatcacggatctggctctggatctggtatcgagggaaggccttataatggaactggatccgcatgcgagctcatgaaaaccctgaaacaagcagagtcctacattaagagtaaagtaaatacaggaactgattttgatggtttatatgggtatcagtgtatggacttagcagtagattatatttaccatgtaacagatggtaaaataagaatgtggggtaatgctaaggatgcgataaataactcttttggtggtactgctacggtatataaaaactaccctgcttttagacctaagtacggtgatgtagtcgtatggactactggtaattttgcaacttatggtcatatcgcaatagttactaaccctgacccttatggagaccttcaatatgttacagttcttgaacaaaactggaacggtaacgggatttataaaaccgagttagctacaatcagaacacacgattacacaggaattacacattttattagacctaactttgctactgaatcaagtgtaaaaaagaaagatacaaagaaaaaaccaaaaccatcaaatagagatggaataaataaagataaaattgtatatgatagaactaatattaattacaattggaaacagaataaagatggcatttggtataaagctgaacatgcttcgttcacagtgacagcaccagagggaattatcacaagatacaaaggtccttggactggtcacccacaagctggtgtattacaaaaaggtcaaacgattaaatatgatgaggttcaaaaatttgacggtcatgtttgggtatcgtgggaaacgtttgagggcgaaactgtatacatgccggtacgcacatgggacgctaaaactggtaaagttggtaagttgtggggcgaaattaaataa

SEQ ID NO: 38 - protein, 308 aa, Artificial Sequence
  artificial construct
MRGSHHHHHHGSGSGSGIEGRPYNGTGSACELMKTLKQAESYIKSKVNTGTDFDGLYGYQCMDLAVDYIYHVTDGKIRMWGNAKDAINNSFGGTATVYKNYPAFRPKYGDVVVWTTGNFATYGHIAIVTNPDPYGDLQYVTVLEQNWNGNGIYKTELATIRTHDYTGITHFIRPNFATESSVKKKDTKKKPKPSNRDGINKDKIVYDRTNINYNWKQNKDGIWYKAEHASFTVTAPEGIITRYKGPWTGHPQAGVLQKGQTIKYDEVQKFDGHVWVSWETFEGETVYMPVRTWDAKTGKVGKLWGEIK

SEQ ID NO: 39 - DNA, 921 bp, Artificial Sequence
  artificial construct
atgagaggatcgcatcaccatcaccatcacggatctggctctggatctggtatcgagggaaggccttataatggaactggatccgcatgcgagctcatgaaaaccctgaaacaagcagagtcctacattaagagtaaagtaaatacaggaactgattttgatggtttatatgggtatcagtgtatggacttagcagtagattatatttaccatgtaacagatggtaaaataagaatgtggggtaatgctaaggatgcgataaataactcttttggtggtactgctacggtatataaaaactaccctgcttttagacctaagtacggtgatgtagtcgtatggactactggtaattttgcaacttatggtcatatcgcaatagttactaaccctgacccttatggagaccttcaatatgttacagttcttgaacaaaactggaacggtaacgggatttataaaaccgagttagctacaatcagaacacacgattacacaggaattacacattttattagacctaactttgctactgaatcaagtgtaaaaaagaaagatacaaagaaaaaaccaaaaccatcaaatagagatggaataaataaagataaaattgtatatgatagaactaatattaattacaattggaaaacaaacaaatatggcacactatataaatcagagtcagctagcttcacacctaatacagatataataacaagaacgactggtccatttagaagcatgccgcagtcaggagtcttaaaagcaggtcaaacaattcattatgatgaagtgatgaaacaagacggtcatgtttgggtaggttatacaggtaacagtggccaacgtatttacttgcctgtaagaacatggaataaatctactaatactttaggtgttctttggggaactataaagtaa

SEQ ID NO: 40 - protein, 306 aa, Artificial Sequence
  artificial construct
MRGSHHHHHHGSGSGSGIEGRPYNGTGSACELMKTLKQAESYIKSKVNTGTDFDGLYGYQCMDLAVDYIYHVTDGKIRMWGNAKDAINNSFGGTATVYKNYPAFRPKYGDVVVWTTGNFATYGHIAIVTNPDPYGDLQYVTVLEQNWNGNGIYKTELATIRTHDYTGITHFIRPNFATESSVKKKDTKKKPKPSNRDGINKDKIVYDRTNINYNWKTNKYGTLYKSESASFTPNTDIITRTTGPFRSMPQSGVLKAGQTIHYDEVMKQDGHVWVGYTGNSGQRIYLPVRTWNKSTNTLGVLWGTIK

SEQ ID NO: 41 - DNA, 927 bp, Artificial Sequence
  artificial construct
atgagaggatcgcatcaccatcaccatcacggatctggctctggatctggtatcgagggaaggccttataatggaactggatccgcatgcgagctcatgaaaaccctgaaacaagcagagtcctacattaagagtaaagtaaatacaggaactgattttgatggtttatatgggtatcagtgtatggacttagcagtagattatatttaccatgtaacagatggtaaaataagaatgtggggtaatgctaaggatgcgataaataactcttttggtggtactgctacggtatataaaaactaccctgcttttagacctaagtacggtgatgtagtcgtatggactactggtaattttgcaacttatggtcatatcgcaatagttactaaccctgacccttatggagaccttcaatatgttacagttcttgaacaaaactggaacggtaacgggatttataaaaccgagttagctacaatcagaacacacgattacacaggaattacacattttattagacctaactttgctactgaatcaagtgtaaaaaagaaagatacaaagaaaaaaccaaaaccatcaaatagagatggaataaataaagataaaattgtatatgatagaactaatattaattacaatggtaaatctgcaagtaaaataacagttggaagtaaagcgccttataaccttaaatggtcaaaaggtgcttattttaatgcgaaaatcgacggcttaggtgctacttcagccactagatacggtgataatcgtactaactatagattcgatgttggacaggctgtatacgcgcctggaacattaatatatgtgtttgaaattatagatggttggtgtcgcatttattggaacaatcataatgagtggatatggcatgagagattgattgtgaaagaagtgttttaa

SEQ ID NO: 42 - protein, 308 aa, Artificial Sequence
  artificial construct
MRGSHHHHHHGSGSGSGIEGRPYNGTGSACELMKTLKQAESYIKSKVNTGTDFDGLYGYQCMDLAVDYIYHVTDGKIRMWGNAKDAINNSFGGTATVYKNYPAFRPKYGDVVVWTTGNFATYGHIAIVTNPDPYGDLQYVTVLEQNWNGNGIYKTELATIRTHDYTGITHFIRPNFATESSVKKKDTKKKPKPSNRDGINKDKIVYDRTNINYNGKSASKITVGSKAPYNLKWSKGAYFNAKIDGLGATSATRYGDNRTNYRFDVGQAVYAPGTLIYVFEIIDGWCRIYWNNHNEWIWHERLIVKEVF

SEQ ID NO: 43 - DNA, 843 bp, Artificial Sequence
  artificial construct
atgagaggatcgcatcaccatcaccatcacggatctggctctggatctggtatcgagggaaggccttataatggaactggatccgcatgcgagctcgctgcaacacatgaacattcagcacaatggttgaataattacaaaaaaggatatggttacggtccttatccattaggtataaatggcggtatgcactacggagttgatttttttatgaatattggaacaccagtaaaagctatttcaagcggaaaaatagttgaagctggttggagtaattacggaggaggtaatcaaataggtcttattgaaaatgatggagtgcatagacaatggtatatgcatctaagtaaatataatgttaaagtaggagattatgtcaaagctggtcaaataatcggttggtctggaagcactggttattctacagcaccacatttacacttccaaagaatggttaattcattttcaaattcaactgcccaagatccaatgcctttcttaaagagcgcaggatatggaaaagcaggtggtacagtaactccaacgccgaatacaggttggaaacagaataaagatggcatttggtataaagctgaacatgcttcgttcacagtgacagcaccagagggaattatcacaagatacaaaggtccttggactggtcacccacaagctggtgtattacaaaaaggtcaaacgattaaatatgatgaggttcaaaaatttgacggtcatgtttgggtatcgtgggaaacgtttgagggcgaaactgtatacatgccggtacgcacatgggacgctaaaactggtaaagttggtaagttgtggggcgaaattaaataa

SEQ ID NO: 44 - protein, 280 aa, Artificial Sequence
  artificial construct
MRGSHHHHHHGSGSGSGIEGRPYNGTGSACELAATHEHSAQWLNNYKKGYGYGPYPLGINGGMHYGVDFFMNIGTPVKAISSGKIVEAGWSNYGGGNQIGLIENDGVHRQWYMHLSKYNVKVGDYVKAGQIIGWSGSTGYSTAPHLHFQRMVNSFSNSTAQDPMPFLKSAGYGKAGGTVTPTPNTGWKQNKDGIWYKAEHASFTVTAPEGIITRYKGPWTGHPQAGVLQKGQTIKYDEVQKFDGHVWVSWETFEGETVYMPVRTWDAKTGKVGKLWGEIK

SEQ ID NO: 45 - DNA, 837 bp, Artificial Sequence
  artificial construct
atgagaggatcgcatcaccatcaccatcacggatctggctctggatctggtatcgagggaaggccttataatggaactggatccgcatgcgagctcgctgcaacacatgaacattcagcacaatggttgaataattacaaaaaaggatatggttacggtccttatccattaggtataaatggcggtatgcactacggagttgatttttttatgaatattggaacaccagtaaaagctatttcaagcggaaaaatagttgaagctggttggagtaattacggaggaggtaatcaaataggtcttattgaaaatgatggagtgcatagacaatggtatatgcatctaagtaaatataatgttaaagtaggagattatgtcaaagctggtcaaataatcggttggtctggaagcactggttattctacagcaccacatttacacttccaaagaatggttaattcattttcaaattcaactgcccaagatccaatgcctttcttaaagagcgcaggatatggaaaagcaggtggtacagtaactccaacgccgaatacaggttggaaaacaaacaaatatggcacactatataaatcagagtcagctagcttcacacctaatacagatataataacaagaacgactggtccatttagaagcatgccgcagtcaggagtcttaaaagcaggtcaaacaattcattatgatgaagtgatgaaacaagacggtcatgtttgggtaggttatacaggtaacagtggccaacgtatttacttgcctgtaagaacatggaataaatctactaatactttaggtgttctttggggaactataaagtaa

SEQ ID NO: 46 - protein, 278 aa, Artificial Sequence
  artificial construct
MRGSHHHHHHGSGSGSGIEGRPYNGTGSACELAATHEHSAQWLNNYKKGYGYGPYPLGINGGMHYGVDFFMNIGTPVKAISSGKIVEAGWSNYGGGNQIGLIENDGVHRQWYMHLSKYNVKVGDYVKAGQIIGWSGSTGYSTAPHLHFQRMVNSFSNSTAQDPMPFLKSAGYGKAGGTVTPTPNTGWKTNKYGTLYKSESASFTPNTDIITRTTGPFRSMPQSGVLKAGQTIHYDEVMKQDGHVWVGYTGNSGQRIYLPVRTWNKSTNTLGVLWGTIK

SEQ ID NO: 47 - DNA, 843 bp, Artificial Sequence
  artificial construct
atgagaggatcgcatcaccatcaccatcacggatctggctctggatctggtatcgagggaaggccttataatggaactggatccgcatgcgagctcgctgcaacacatgaacattcagcacaatggttgaataattacaaaaaaggatatggttacggtccttatccattaggtataaatggcggtatgcactacggagttgatttttttatgaatattggaacaccagtaaaagctatttcaagcggaaaaatagttgaagctggttggagtaattacggaggaggtaatcaaataggtcttattgaaaatgatggagtgcatagacaatggtatatgcatctaagtaaatataatgttaaagtaggagattatgtcaaagctggtcaaataatcggttggtctggaagcactggttattctacagcaccacatttacacttccaaagaatggttaattcattttcaaattcaactgcccaagatccaatgcctttcttaaagagcgcaggatatggaaaagcaggtggtacagtaactccaacgccgaatacaggtggtaaatctgcaagtaaaataacagttggaagtaaagcgccttataaccttaaatggtcaaaaggtgcttattttaatgcgaaaatcgacggcttaggtgctacttcagccactagatacggtgataatcgtactaactatagattcgatgttggacaggctgtatacgcgcctggaacattaatatatgtgtttgaaattatagatggttggtgtcgcatttattggaacaatcataatgagtggatatggcatgagagattgattgtgaaagaagtgttttaa

SEQ ID NO: 48 - protein, 280 aa, Artificial Sequence
  artificial construct
MRGSHHHHHHGSGSGSGIEGRPYNGTGSACELAATHEHSAQWLNNYKKGYGYGPYPLGINGGMHYGVDFFMNIGTPVKAISSGKIVEAGWSNYGGGNQIGLIENDGVHRQWYMHLSKYNVKVGDYVKAGQIIGWSGSTGYSTAPHLHFQRMVNSFSNSTAQDPMPFLKSAGYGKAGGTVTPTPNTGGKSASKITVGSKAPYNLKWSKGAYFNAKIDGLGATSATRYGDNRTNYRFDVGQAVYAPGTLIYVFEIIDGWCRIYWNNHNEWIWHERLIVKEVF

SEQ ID NO: 49 - DNA, 1755 bp, Artificial Sequence
  artificial construct
atgagaggatcgcatcaccatcaccatcacggatctggctctggatctggtatcgagggaagggcaaagaaagatgaaaaatcacaagtatgtagtggtttggctatggaaaaatatgacattacaaatttaaatgctaaacaagataaatcaaagaatgggagcgtgaaagagttgaaacatatctattcaaaccatattaaaggtaacaagattacagcaccaaaacctagtattcaaggtgtggtcatccacaatgattatggtagtatgacacctagtcaatacttaccatggttatatgcacgtgagaataacggtacacacgttaacggttgggctagtgtttatgcaaatagaaacgaagtgctttggtatcatccgacagactacgtagagtggcattgtggtaatcaatgggcaaatgctaacttaatcggatttgaagtgtgtgagtcgtatcctggtagaatctcggacaaattattcttagaaaatgaagaagcgacattgaaagtagctgcggatgtgatgaagtcgtacggattaccagttaatcgcaacactgtacgtctgcataacgaattcttcggaacttcttgtccacatcgttcgtgggacttgcatgttggcaaaggtgagccttacacaactactaatattaataaaatgaaagactacttcatcaaacgcatcaaacattattatgacggtgagctcgcaaagaaagatgaaaaatcacaagtatgtagtggtttggctatggaaaaatatgacattacaaatttaaatgctaaacaagataaatcaaagaatgggagcgtgaaagagttgaaacatatctattcaaaccatattaaaggtaacaagattacagcaccaaaacctagtattcaaggtgtggtcatccacaatgattatggtagtatgacacctagtcaatacttaccatggttatatgcacgtgagaataacggtacacacgttaacggttgggctagtgtttatgcaaatagaaacgaagtgctttggtatcatccgacagactacgtagagtggcattgtggtaatcaatgggcaaatgctaacttaatcggatttgaagtgtgtgagtcgtatcctggtagaatctcggacaaattattcttagaaaatgaagaagcgacattgaaagtagctgcggatgtgatgaagtcgtacggattaccagttaatcgcaacactgtacgtctgcataacgaattcttcggaacttcttgtccacatcgttcgtgggacttgcatgttggcaaaggtgagccttacacaactactaatattaataaaatgaaagactacttcatcaaacgcatcaaacattattatgacggtggaaagctagaagtaagcaaagcagcaactatcaaacaatctgacgttaagcaagaagttaaaaagcaagaagcaaaacaaattgtgaaagcaacagattggaaacagaataaagatggcatttggtataaagctgaacatgcttcgttcacagtgacagcaccagagggaattatcacaagatacaaaggtccttggactggtcacccacaagctggtgtattacaaaaaggtcaaacgattaaatatgatgaggttcaaaaatttgacggtcatgtttgggtatcgtgggaaacgtttgagggcgaaactgtatacatgccggtacgcacatgggacgctaaaactggtaaagttggtaagttgtggggcgaaattaaataa

SEQ ID NO: 50 - protein, 584 aa, Artificial Sequence
  artificial construct
MRGSHHHHHHGSGSGSGIEGRAKKDEKSQVCSGLAMEKYDITNLNAKQDKSKNGSVKELKHIYSNHIKGNKITAPKPSIQGVVIHNDYGSMTPSQYLPWLYARENNGTHVNGWASVYANRNEVLWYHPTDYVEWHCGNQWANANLIGFEVCESYPGRISDKLFLENEEATLKVAADVMKSYGLPVNRNTVRLHNEFFGTSCPHRSWDLHVGKGEPYTTTNINKMKDYFIKRIKHYYDGELAKKDEKSQVCSGLAMEKYDITNLNAKQDKSKNGSVKELKHIYSNHIKGNKITAPKPSIQGVVIHNDYGSMTPSQYLPWLYARENNGTHVNGWASVYANRNEVLWYHPTDYVEWHCGNQWANANLIGFEVCESYPGRISDKLFLENEEATLKVAADVMKSYGLPVNRNTVRLHNEFFGTSCPHRSWDLHVGKGEPYTTTNINKMKDYFIKRIKHYYDGGKLEVSKAATIKQSDVKQEVKKQEAKQIVKATDWKQNKDGIWYKAEHASFTVTAPEGIITRYKGPWTGHPQAGVLQKGQTIKYDEVQKFDGHVWVSWETFEGETVYMPVRTWDAKTGKVGKLWGEIK

SEQ ID NO: 51 - DNA, 1749 bp, Artificial Sequence
  artificial construct
atgagaggatcgcatcaccatcaccatcacggatctggctctggatctggtatcgagggaagggcaaagaaagatgaaaaatcacaagtatgtagtggtttggctatggaaaaatatgacattacaaatttaaatgctaaacaagataaatcaaagaatgggagcgtgaaagagttgaaacatatctattcaaaccatattaaaggtaacaagattacagcaccaaaacctagtattcaaggtgtggtcatccacaatgattatggtagtatgacacctagtcaatacttaccatggttatatgcacgtgagaataacggtacacacgttaacggttgggctagtgtttatgcaaatagaaacgaagtgctttggtatcatccgacagactacgtagagtggcattgtggtaatcaatgggcaaatgctaacttaatcggatttgaagtgtgtgagtcgtatcctggtagaatctcggacaaattattcttagaaaatgaagaagcgacattgaaagtagctgcggatgtgatgaagtcgtacggattaccagttaatcgcaacactgtacgtctgcataacgaattcttcggaacttcttgtccacatcgttcgtgggacttgcatgttggcaaaggtgagccttacacaactactaatattaataaaatgaaagactacttcatcaaacgcatcaaacattattatgacggtgagctcgcaaagaaagatgaaaaatcacaagtatgtagtggtttggctatggaaaaatatgacattacaaatttaaatgctaaacaagataaatcaaagaatgggagcgtgaaagagttgaaacatatctattcaaaccatattaaaggtaacaagattacagcaccaaaacctagtattcaaggtgtggtcatccacaatgattatggtagtatgacacctagtcaatacttaccatggttatatgcacgtgagaataacggtacacacgttaacggttgggctagtgtttatgcaaatagaaacgaagtgctttggtatcatccgacagactacgtagagtggcattgtggtaatcaatgggcaaatgctaacttaatcggatttgaagtgtgtgagtcgtatcctggtagaatctcggacaaattattcttagaaaatgaagaagcgacattgaaagtagctgcggatgtgatgaagtcgtacggattaccagttaatcgcaacactgtacgtctgcataacgaattcttcggaacttcttgtccacatcgttcgtgggacttgcatgttggcaaaggtgagccttacacaactactaatattaataaaatgaaagactacttcatcaaacgcatcaaacattattatgacggtggaaagctagaagtaagcaaagcagcaactatcaaacaatctgacgttaagcaagaagttaaaaagcaagaagcaaaacaaattgtgaaagcaacagattggaaaacaaacaaatatggcacactatataaatcagagtcagctagcttcacacctaatacagatataataacaagaacgactggtccatttagaagcatgccgcagtcaggagtcttaaaagcaggtcaaacaattcattatgatgaagtgatgaaacaagacggtcatgtttgggtaggttatacaggtaacagtggccaacgtatttacttgcctgtaagaacatggaataaatctactaatactttaggtgttctttggggaactataaagtaa

SEQ ID NO: 52 - protein, 582 aa, Artificial Sequence
  artificial construct
MRGSHHHHHHGSGSGSGIEGRAKKDEKSQVCSGLAMEKYDITNLNAKQDKSKNGSVKELKHIYSNHIKGNKITAPKPSIQGVVIHNDYGSMTPSQYLPWLYARENNGTHVNGWASVYANRNEVLWYHPTDYVEWHCGNQWANANLIGFEVCESYPGRISDKLFLENEEATLKVAADVMKSYGLPVNRNTVRLHNEFFGTSCPHRSWDLHVGKGEPYTTTNINKMKDYFIKRIKHYYDGELAKKDEKSQVCSGLAMEKYDITNLNAKQDKSKNGSVKELKHIYSNHIKGNKITAPKPSIQGVVIHNDYGSMTPSQYLPWLYARENNGTHVNGWASVYANRNEVLWYHPTDYVEWHCGNQWANANLIGFEVCESYPGRISDKLFLENEEATLKVAADVMKSYGLPVNRNTVRLHNEFFGTSCPHRSWDLHVGKGEPYTTTNINKMKDYFIKRIKHYYDGGKLEVSKAATIKQSDVKQEVKKQEAKQIVKATDWKTNKYGTLYKSESASFTPNTDIITRTTGPFRSMPQSGVLKAGQTIHYDEVMKQDGHVWVGYTGNSGQRIYLPVRTWNKSTNTLGVLWGTIK

SEQ ID NO: 53 - DNA, 1755 bp, Artificial Sequence
  artificial construct
atgagaggatcgcatcaccatcaccatcacggatctggctctggatctggtatcgagggaagggcaaagaaagatgaaaaatcacaagtatgtagtggtttggctatggaaaaatatgacattacaaatttaaatgctaaacaagataaatcaaagaatgggagcgtgaaagagttgaaacatatctattcaaaccatattaaaggtaacaagattacagcaccaaaacctagtattcaaggtgtggtcatccacaatgattatggtagtatgacacctagtcaatacttaccatggttatatgcacgtgagaataacggtacacacgttaacggttgggctagtgtttatgcaaatagaaacgaagtgctttggtatcatccgacagactacgtagagtggcattgtggtaatcaatgggcaaatgctaacttaatcggatttgaagtgtgtgagtcgtatcctggtagaatctcggacaaattattcttagaaaatgaagaagcgacattgaaagtagctgcggatgtgatgaagtcgtacggattaccagttaatcgcaacactgtacgtctgcataacgaattcttcggaacttcttgtccacatcgttcgtgggacttgcatgttggcaaaggtgagccttacacaactactaatattaataaaatgaaagactacttcatcaaacgcatcaaacattattatgacggtgagctcgcaaagaaagatgaaaaatcacaagtatgtagtggtttggctatggaaaaatatgacattacaaatttaaatgctaaacaagataaatcaaagaatgggagcgtgaaagagttgaaacatatctattcaaaccatattaaaggtaacaagattacagcaccaaaacctagtattcaaggtgtggtcatccacaatgattatggtagtatgacacctagtcaatacttaccatggttatatgcacgtgagaataacggtacacacgttaacggttgggctagtgtttatgcaaatagaaacgaagtgctttggtatcatccgacagactacgtagagtggcattgtggtaatcaatgggcaaatgctaacttaatcggatttgaagtgtgtgagtcgtatcctggtagaatctcggacaaattattcttagaaaatgaagaagcgacattgaaagtagctgcggatgtgatgaagtcgtacggattaccagttaatcgcaacactgtacgtctgcataacgaattcttcggaacttcttgtccacatcgttcgtgggacttgcatgttggcaaaggtgagccttacacaactactaatattaataaaatgaaagactacttcatcaaacgcatcaaacattattatgacggtggaaagctagaagtaagcaaagcagcaactatcaaacaatctgacgttaagcaagaagttaaaaagcaagaagcaaaacaaattgtgaaagcaacagatggtaaatctgcaagtaaaataacagttggaagtaaagcgccttataaccttaaatggtcaaaaggtgcttattttaatgcgaaaatcgacggcttaggtgctacttcagccactagatacggtgataatcgtactaactatagattcgatgttggacaggctgtatacgcgcctggaacattaatatatgtgtttgaaattatagatggttggtgtcgcatttattggaacaatcataatgagtggatatggcatgagagattgattgtgaaagaagtgttttaa

SEQ ID NO: 54 - protein, 584 aa, Artificial Sequence
  artificial construct
MRGSHHHHHHGSGSGSGIEGRAKKDEKSQVCSGLAMEKYDITNLNAKQDKSKNGSVKELKHIYSNHIKGNKITAPKPSIQGVVIHNDYGSMTPSQYLPWLYARENNGTHVNGWASVYANRNEVLWYHPTDYVEWHCGNQWANANLIGFEVCESYPGRISDKLFLENEEATLKVAADVMKSYGLPVNRNTVRLHNEFFGTSCPHRSWDLHVGKGEPYTTTNINKMKDYFIKRIKHYYDGELAKKDEKSQVCSGLAMEKYDITNLNAKQDKSKNGSVKELKHIYSNHIKGNKITAPKPSIQGVVIHNDYGSMTPSQYLPWLYARENNGTHVNGWASVYANRNEVLWYHPTDYVEWHCGNQWANANLIGFEVCESYPGRISDKLFLENEEATLKVAADVMKSYGLPVNRNTVRLHNEFFGTSCPHRSWDLHVGKGEPYTTTNINKMKDYFIKRIKHYYDGGKLEVSKAATIKQSDVKQEVKKQEAKQIVKATDGKSASKITVGSKAPYNLKWSKGAYFNAKIDGLGATSATRYGDNRTNYRFDVGQAVYAPGTLIYVFEIIDGWCRIYWNNHNEWIWHERLIVKEVF

SEQ ID NO: 55 - DNA, 1533 bp, Artificial Sequence
  artificial construct
atgagaggatcgcatcaccatcaccatcacggatctggctctggatctggtatcgagggaaggatggctaagactcaagcagaaataaataaacgtttagatgcttatgcaaaaggaacagtagatagcccttacagagttaaaaaagctacaagttatgacccatcatttggtgtaatggaagcaggagccattgatgcagatggttactatcacgctcagtgtcaagaccttattacagactatgttttatggttaacagataataaagttagaacttggggtaatgctaaagaccaaattaaacagagttatggtactggatttaaaatacatgaaaataaaccttctactgtacctaaaaaaggttggattgcggtatttacatccggtagttatgaacagtggggtcacataggtattgtatatgatggaggtaatacttctacatttactattttagagcaaaactggaatggttatgctaataaaaaacctacaaaacgtgtagataattattacggattaactcacttcattgaaatacctgtaaaagcaggaactactgttaaaaaagaaacagctaagaaaagcgcaagtaaaacgcctgcacctaaaaagaaagcaacactaaaagtttctaagaatgagctcatggctaagactcaagcagaaataaataaacgtttagatgcttatgcaaaaggaacagtagatagcccttacagagttaaaaaagctacaagttatgacccatcatttggtgtaatggaagcaggagccattgatgcagatggttactatcacgctcagtgtcaagaccttattacagactatgttttatggttaacagataataaagttagaacttggggtaatgctaaagaccaaattaaacagagttatggtactggatttaaaatacatgaaaataaaccttctactgtacctaaaaaaggttggattgcggtatttacatccggtagttatgaacagtggggtcacataggtattgtatatgatggaggtaatacttctacatttactattttagagcaaaactggaatggttatgctaataaaaaacctacaaaacgtgtagataattattacggattaactcacttcattgaaatacctgtaaaagcaggaaagctagaagtaagcaaagcagcaactatcaaacaatctgacgttaagcaagaagttaaaaagcaagaagcaaaacaaattgtgaaagcaacagattggaaacagaataaagatggcatttggtataaagctgaacatgcttcgttcacagtgacagcaccagagggaattatcacaagatacaaaggtccttggactggtcacccacaagctggtgtattacaaaaaggtcaaacgattaaatatgatgaggttcaaaaatttgacggtcatgtttgggtatcgtgggaaacgtttgagggcgaaactgtatacatgccggtacgcacatgggacgctaaaactggtaaagttggtaagttgtggggcgaaattaaataa

SEQ ID NO: 56 - protein, 510 aa, Artificial Sequence
  artificial construct
MRGSHHHHHHGSGSGSGIEGRMAKTQAEINKRLDAYAKGTVDSPYRVKKATSYDPSFGVMEAGAIDADGYYHAQCQDLITDYVLWLTDNKVRTWGNAKDQIKQSYGTGFKIHENKPSTVPKKGWIAVFTSGSYEQWGHIGIVYDGGNTSTFTILEQNWNGYANKKPTKRVDNYYGLTHFIEIPVKAGTTVKKETAKKSASKTPAPKKKATLKVSKNELMAKTQAEINKRLDAYAKGTVDSPYRVKKATSYDPSFGVMEAGAIDADGYYHAQCQDLITDYVLWLTDNKVRTWGNAKDQIKQSYGTGFKIHENKPSTVPKKGWIAVFTSGSYEQWGHIGIVYDGGNTSTFTILEQNWNGYANKKPTKRVDNYYGLTHFIEIPVKAGKLEVSKAATIKQSDVKQEVKKQEAKQIVKATDWKQNKDGIWYKAEHASFTVTAPEGIITRYKGPWTGHPQAGVLQKGQTIKYDEVQKFDGHVWVSWETFEGETVYMPVRTWDAKTGKVGKLWGEIK

SEQ ID NO: 57 - DNA, 1470 bp, Artificial Sequence
  artificial construct
atgagaggatcgcatcaccatcaccatcacggatctggctctggatctggtatcgagggaaggatggctaagactcaagcagaaataaataaacgtttagatgcttatgcaaaaggaacagtagatagcccttacagagttaaaaaagctacaagttatgacccatcatttggtgtaatggaagcaggagccattgatgcagatggttactatcacgctcagtgtcaagaccttattacagactatgttttatggttaacagataataaagttagaacttggggtaatgctaaagaccaaattaaacagagttatggtactggatttaaaatacatgaaaataaaccttctactgtacctaaaaaaggttggattgcggtatttacatccggtagttatgaacagtggggtcacataggtattgtatatgatggaggtaatacttctacatttactattttagagcaaaactggaatggttatgctaataaaaaacctacaaaacgtgtagataattattacggattaactcacttcattgaaatacctgtaaaagcaggaactactgttaaaaaagaaacagctaagaaaagcgcaagtaaaacgcctgcacctaaaaagaaagcaacactaaaagtttctaagaatgagctcatggctaagactcaagcagaaataaataaacgtttagatgcttatgcaaaaggaacagtagatagcccttacagagttaaaaaagctacaagttatgacccatcatttggtgtaatggaagcaggagccattgatgcagatggttactatcacgctcagtgtcaagaccttattacagactatgttttatggttaacagataataaagttagaacttggggtaatgctaaagaccaaattaaacagagttatggtactggatttaaaatacatgaaaataaaccttctactgtacctaaaaaaggttggattgcggtatttacatccggtagttatgaacagtggggtcacataggtattgtatatgatggaggtaatacttctacatttactattttagagcaaaactggaatggttatgctaataaaaaacctacaaaacgtgtagataattattacggattaactcacttcattgaaatacctgtaaaagcaggaaaagcaggtggtacagtaactccaacgccgaatacaggttggaaaacaaacaaatatggcacactatataaatcagagtcagctagcttcacacctaatacagatataataacaagaacgactggtccatttagaagcatgccgcagtcaggagtcttaaaagcaggtcaaacaattcattatgatgaagtgatgaaacaagacggtcatgtttgggtaggttatacaggtaacagtggccaacgtatttacttgcctgtaagaacatggaataaatctactaatactttaggtgttctttggggaactataaagtaa

SEQ ID NO: 58 - protein, 489 aa, Artificial Sequence
  artificial construct
MRGSHHHHHHGSGSGSGIEGRMAKTQAEINKRLDAYAKGTVDSPYRVKKATSYDPSFGVMEAGAIDADGYYHAQCQDLITDYVLWLTDNKVRTWGNAKDQIKQSYGTGFKIHENKPSTVPKKGWIAVFTSGSYEQWGHIGIVYDGGNTSTFTILEQNWNGYANKKPTKRVDNYYGLTHFIEIPVKAGTTVKKETAKKSASKTPAPKKKATLKVSKNELMAKTQAEINKRLDAYAKGTVDSPYRVKKATSYDPSFGVMEAGAIDADGYYHAQCQDLITDYVLWLTDNKVRTWGNAKDQIKQSYGTGFKIHENKPSTVPKKGWIAVFTSGSYEQWGHIGIVYDGGNTSTFTILEQNWNGYANKKPTKRVDNYYGLTHFIEIPVKAGKAGGTVTPTPNTGWKTNKYGTLYKSESASFTPNTDIITRTTGPFRSMPQSGVLKAGQTIHYDEVMKQDGHVWVGYTGNSGQRIYLPVRTWNKSTNTLGVLWGTIK

SEQ ID NO: 59 - DNA, 1524 bp, Artificial Sequence
  artificial construct
atgagaggatcgcatcaccatcaccatcacggatctggctctggatctggtatcgagggaaggatggctaagactcaagcagaaataaataaacgtttagatgcttatgcaaaaggaacagtagatagcccttacagagttaaaaaagctacaagttatgacccatcatttggtgtaatggaagcaggagccattgatgcagatggttactatcacgctcagtgtcaagaccttattacagactatgttttatggttaacagataataaagttagaacttggggtaatgctaaagaccaaattaaacagagttatggtactggatttaaaatacatgaaaataaaccttctactgtacctaaaaaaggttggattgcggtatttacatccggtagttatgaacagtggggtcacataggtattgtatatgatggaggtaatacttctacatttactattttagagcaaaactggaatggttatgctaataaaaaacctacaaaacgtgtagataattattacggattaactcacttcattgaaatacctgtaaaagcaggaactactgttaaaaaagaaacagctaagaaaagcgcaagtaaaacgcctgcacctaaaaagaaagcaacactaaaagtttctaagaatgagctcatggctaagactcaagcagaaataaataaacgtttagatgcttatgcaaaaggaacagtagatagcccttacagagttaaaaaagctacaagttatgacccatcatttggtgtaatggaagcaggagccattgatgcagatggttactatcacgctcagtgtcaagaccttattacagactatgttttatggttaacagataataaagttagaacttggggtaatgctaaagaccaaattaaacagagttatggtactggatttaaaatacatgaaaataaaccttctactgtacctaaaaaaggttggattgcggtatttacatccggtagttatgaacagtggggtcacataggtattgtatatgatggaggtaatacttctacatttactattttagagcaaaactggaatggttatgctaataaaaaacctacaaaacgtgtagataattattacggattaactcacttcattgaaatacctgtaaaagcaggaactactgttaaaaaagaaacagctaagaaaagcgcaagtaaaacgcctgcacctaaaaagaaagcaacactaaaagtttctaagaatggtaaatctgcaagtaaaataacagttggaagtaaagcgccttataaccttaaatggtcaaaaggtgcttattttaatgcgaaaatcgacggcttaggtgctacttcagccactagatacggtgataatcgtactaactatagattcgatgttggacaggctgtatacgcgcctggaacattaatatatgtgtttgaaattatagatggttggtgtcgcatttattggaacaatcataatgagtggatatggcatgagagattgattgtgaaagaagtgttttaa

SEQ ID NO: 60 - protein, 507 aa, Artificial Sequence
  artificial construct
MRGSHHHHHHGSGSGSGIEGRMAKTQAEINKRLDAYAKGTVDSPYRVKKATSYDPSFGVMEAGAIDADGYYHAQCQDLITDYVLWLTDNKVRTWGNAKDQIKQSYGTGFKIHENKPSTVPKKGWIAVFTSGSYEQWGHIGIVYDGGNTSTFTILEQNWNGYANKKPTKRVDNYYGLTHFIEIPVKAGTTVKKETAKKSASKTPAPKKKATLKVSKNELMAKTQAEINKRLDAYAKGTVDSPYRVKKATSYDPSFGVMEAGAIDADGYYHAQCQDLITDYVLWLTDNKVRTWGNAKDQIKQSYGTGFKIHENKPSTVPKKGWIAVFTSGSYEQWGHIGIVYDGGNTSTFTILEQNWNGYANKKPTKRVDNYYGLTHFIEIPVKAGTTVKKETAKKSASKTPAPKKKATLKVSKNGKSASKITVGSKAPYNLKWSKGAYFNAKIDGLGATSATRYGDNRTNYRFDVGQAVYAPGTLIYVFEIIDGWCRIYWNNHNEWIWHERLIVKEVF

SEQ ID NO: 61 - DNA, 1446 bp, Artificial Sequence
  artificial construct
atgagaggatcgcatcaccatcaccatcacggatctggctctggatctggtatcgagggaaggatgaaaaccctgaaacaagcagagtcctacattaagagtaaagtaaatacaggaactgattttgatggtttatatgggtatcagtgtatggacttagcagtagattatatttaccatgtaacagatggtaaaataagaatgtggggtaatgctaaggatgcgataaataactcttttggtggtactgctacggtatataaaaactaccctgcttttagacctaagtacggtgatgtagtcgtatggactactggtaattttgcaacttatggtcatatcgcaatagttactaaccctgacccttatggagaccttcaatatgttacagttcttgaacaaaactggaacggtaacgggatttataaaaccgagttagctacaatcagaacacacgattacacaggaattacacattttattagacctaactttgctactgaatcaagtgtaaaaaagaaagatacaaagaaaaaaccaaaaccatcaaatagagatggaataaataaagataaaattgtatatgatagaactaatattaattacaatgagctcatgaaaaccctgaaacaagcagagtcctacattaagagtaaagtaaatacaggaactgattttgatggtttatatgggtatcagtgtatggacttagcagtagattatatttaccatgtaacagatggtaaaataagaatgtggggtaatgctaaggatgcgataaataactcttttggtggtactgctacggtatataaaaactaccctgcttttagacctaagtacggtgatgtagtcgtatggactactggtaattttgcaacttatggtcatatcgcaatagttactaaccctgacccttatggagaccttcaatatgttacagttcttgaacaaaactggaacggtaacgggatttataaaaccgagttagctacaatcagaacacacgattacacaggaattacacattttattagacctaactttgctactgaatcaagtgtaaaaaagaaagatacaaagaaaaaaccaaaaccatcaaatagagatggaataaataaagataaaattgtatatgatagaactaatattaattacaattggaaacagaataaagatggcatttggtataaagctgaacatgcttcgttcacagtgacagcaccagagggaattatcacaagatacaaaggtccttggactggtcacccacaagctggtgtattacaaaaaggtcaaacgattaaatatgatgaggttcaaaaatttgacggtcatgtttgggtatcgtgggaaacgtttgagggcgaaactgtatacatgccggtacgcacatgggacgctaaaactggtaaagttggtaagttgtggggcgaaattaaataa

SEQ ID NO: 62 - protein, 481 aa, Artificial Sequence
  artificial construct
MRGSHHHHHHGSGSGSGIEGRMKTLKQAESYIKSKVNTGTDFDGLYGYQCMDLAVDYIYHVTDGKIRMWGNAKDAINNSFGGTATVYKNYPAFRPKYGDVVVWTTGNFATYGHIAIVTNPDPYGDLQYVTVLEQNWNGNGIYKTELATIRTHDYTGITHFIRPNFATESSVKKKDTKKKPKPSNRDGINKDKIVYDRTNINYNELMKTLKQAESYIKSKVNTGTDFDGLYGYQCMDLAVDYIYHVTDGKIRMWGNAKDAINNSFGGTATVYKNYPAFRPKYGDVVVWTTGNFATYGHIAIVTNPDPYGDLQYVTVLEQNWNGNGIYKTELATIRTHDYTGITHFIRPNFATESSVKKKDTKKKPKPSNRDGINKDKIVYDRTNINYNWKQNKDGIWYKAEHASFTVTAPEGIITRYKGPWTGHPQAGVLQKGQTIKYDEVQKFDGHVWVSWETFEGETVYMPVRTWDAKTGKVGKLWGEIK

SEQ ID NO: 63 - DNA, 1440 bp, Artificial Sequence
  artificial construct
atgagaggatcgcatcaccatcaccatcacggatctggctctggatctggtatcgagggaaggatgaaaaccctgaaacaagcagagtcctacattaagagtaaagtaaatacaggaactgattttgatggtttatatgggtatcagtgtatggacttagcagtagattatatttaccatgtaacagatggtaaaataagaatgtggggtaatgctaaggatgcgataaataactcttttggtggtactgctacggtatataaaaactaccctgcttttagacctaagtacggtgatgtagtcgtatggactactggtaattttgcaacttatggtcatatcgcaatagttactaaccctgacccttatggagaccttcaatatgttacagttcttgaacaaaactggaacggtaacgggatttataaaaccgagttagctacaatcagaacacacgattacacaggaattacacattttattagacctaactttgctactgaatcaagtgtaaaaaagaaagatacaaagaaaaaaccaaaaccatcaaatagagatggaataaataaagataaaattgtatatgatagaactaatattaattacaatgagctcatgaaaaccctgaaacaagcagagtcctacattaagagtaaagtaaatacaggaactgattttgatggtttatatgggtatcagtgtatggacttagcagtagattatatttaccatgtaacagatggtaaaataagaatgtggggtaatgctaaggatgcgataaataactcttttggtggtactgctacggtatataaaaactaccctgcttttagacctaagtacggtgatgtagtcgtatggactactggtaattttgcaacttatggtcatatcgcaatagttactaaccctgacccttatggagaccttcaatatgttacagttcttgaacaaaactggaacggtaacgggatttataaaaccgagttagctacaatcagaacacacgattacacaggaattacacattttattagacctaactttgctactgaatcaagtgtaaaaaagaaagatacaaagaaaaaaccaaaaccatcaaatagagatggaataaataaagataaaattgtatatgatagaactaatattaattacaattggaaaacaaacaaatatggcacactatataaatcagagtcagctagcttcacacctaatacagatataataacaagaacgactggtccatttagaagcatgccgcagtcaggagtcttaaaagcaggtcaaacaattcattatgatgaagtgatgaaacaagacggtcatgtttgggtaggttatacaggtaacagtggccaacgtatttacttgcctgtaagaacatggaataaatctactaatactttaggtgttctttggggaactataaagtaa

SEQ ID NO: 64 - protein, 479 aa, Artificial Sequence
  artificial construct
MRGSHHHHHHGSGSGSGIEGRMKTLKQAESYIKSKVNTGTDFDGLYGYQCMDLAVDYIYHVTDGKIRMWGNAKDAINNSFGGTATVYKNYPAFRPKYGDVVVWTTGNFATYGHIAIVTNPDPYGDLQYVTVLEQNWNGNGIYKTELATIRTHDYTGITHFIRPNFATESSVKKKDTKKKPKPSNRDGINKDKIVYDRTNINYNELMKTLKQAESYIKSKVNTGTDFDGLYGYQCMDLAVDYIYHVTDGKIRMWGNAKDAINNSFGGTATVYKNYPAFRPKYGDVVVWTTGNFATYGHIAIVTNPDPYGDLQYVTVLEQNWNGNGIYKTELATIRTHDYTGITHFIRPNFATESSVKKKDTKKKPKPSNRDGINKDKIVYDRTNINYNWKTNKYGTLYKSESASFTPNTDIITRTTGPFRSMPQSGVLKAGQTIHYDEVMKQDGHVWVGYTGNSGQRIYLPVRTWNKSTNTLGVLWGTIK

SEQ ID NO: 65 - DNA, 1446 bp, Artificial Sequence
  artificial construct
atgagaggatcgcatcaccatcaccatcacggatctggctctggatctggtatcgagggaaggatgaaaaccctgaaacaagcagagtcctacattaagagtaaagtaaatacaggaactgattttgatggtttatatgggtatcagtgtatggacttagcagtagattatatttaccatgtaacagatggtaaaataagaatgtggggtaatgctaaggatgcgataaataactcttttggtggtactgctacggtatataaaaactaccctgcttttagacctaagtacggtgatgtagtcgtatggactactggtaattttgcaacttatggtcatatcgcaatagttactaaccctgacccttatggagaccttcaatatgttacagttcttgaacaaaactggaacggtaacgggatttataaaaccgagttagctacaatcagaacacacgattacacaggaattacacattttattagacctaactttgctactgaatcaagtgtaaaaaagaaagatacaaagaaaaaaccaaaaccatcaaatagagatggaataaataaagataaaattgtatatgatagaactaatattaattacaatgagctcatgaaaaccctgaaacaagcagagtcctacattaagagtaaagtaaatacaggaactgattttgatggtttatatgggtatcagtgtatggacttagcagtagattatatttaccatgtaacagatggtaaaataagaatgtggggtaatgctaaggatgcgataaataactcttttggtggtactgctacggtatataaaaactaccctgcttttagacctaagtacggtgatgtagtcgtatggactactggtaattttgcaacttatggtcatatcgcaatagttactaaccctgacccttatggagaccttcaatatgttacagttcttgaacaaaactggaacggtaacgggatttataaaaccgagttagctacaatcagaacacacgattacacaggaattacacattttattagacctaactttgctactgaatcaagtgtaaaaaagaaagatacaaagaaaaaaccaaaaccatcaaatagagatggaataaataaagataaaattgtatatgatagaactaatattaattacaatggtaaatctgcaagtaaaataacagttggaagtaaagcgccttataaccttaaatggtcaaaaggtgcttattttaatgcgaaaatcgacggcttaggtgctacttcagccactagatacggtgataatcgtactaactatagattcgatgttggacaggctgtatacgcgcctggaacattaatatatgtgtttgaaattatagatggttggtgtcgcatttattggaacaatcataatgagtggatatggcatgagagattgattgtgaaagaagtgttttaa

SEQ ID NO: 66 - protein, 481 aa, Artificial Sequence
  artificial construct
MRGSHHHHHHGSGSGSGIEGRMKTLKQAESYIKSKVNTGTDFDGLYGYQCMDLAVDYIYHVTDGKIRMWGNAKDAINNSFGGTATVYKNYPAFRPKYGDVVVWTTGNFATYGHIAIVTNPDPYGDLQYVTVLEQNWNGNGIYKTELATIRTHDYTGITHFIRPNFATESSVKKKDTKKKPKPSNRDGINKDKIVYDRTNINYNELMKTLKQAESYIKSKVNTGTDFDGLYGYQCMDLAVDYIYHVTDGKIRMWGNAKDAINNSFGGTATVYKNYPAFRPKYGDVVVWTTGNFATYGHIAIVTNPDPYGDLQYVTVLEQNWNGNGIYKTELATIRTHDYTGITHFIRPNFATESSVKKKDTKKKPKPSNRDGINKDKIVYDRTNINYNGKSASKITVGSKAPYNLKWSKGAYFNAKIDGLGATSATRYGDNRTNYRFDVGQAVYAPGTLIYVFEIIDGWCRIYWNNHNEWIWHERLIVKEVF

SEQ ID NO: 67 - DNA, 1278 bp, Artificial Sequence
  artificial construct
atgagaggatcgcatcaccatcaccatcacggatctggctctggatctggtatcgagggaagggctgcaacacatgaacattcagcacaatggttgaataattacaaaaaaggatatggttacggtccttatccattaggtataaatggcggtatgcactacggagttgatttttttatgaatattggaacaccagtaaaagctatttcaagcggaaaaatagttgaagctggttggagtaattacggaggaggtaatcaaataggtcttattgaaaatgatggagtgcatagacaatggtatatgcatctaagtaaatataatgttaaagtaggagattatgtcaaagctggtcaaataatcggttggtctggaagcactggttattctacagcaccacatttacacttccaaagaatggttaattcattttcaaattcaactgcccaagatccaatgcctttcttaaagagcgcaggatatggaaaagcaggtggtacagtaactccaacgccgaatacaggtgagctcgctgcaacacatgaacattcagcacaatggttgaataattacaaaaaaggatatggttacggtccttatccattaggtataaatggcggtatgcactacggagttgatttttttatgaatattggaacaccagtaaaagctatttcaagcggaaaaatagttgaagctggttggagtaattacggaggaggtaatcaaataggtcttattgaaaatgatggagtgcatagacaatggtatatgcatctaagtaaatataatgttaaagtaggagattatgtcaaagctggtcaaataatcggttggtctggaagcactggttattctacagcaccacatttacacttccaaagaatggttaattcattttcaaattcaactgcccaagatccaatgcctttcttaaagagcgcaggatatggaaaagcaggtggtacagtaactccaacgccgaatacaggttggaaacagaataaagatggcatttggtataaagctgaacatgcttcgttcacagtgacagcaccagagggaattatcacaagatacaaaggtccttggactggtcacccacaagctggtgtattacaaaaaggtcaaacgattaaatatgatgaggttcaaaaatttgacggtcatgtttgggtatcgtgggaaacgtttgagggcgaaactgtatacatgccggtacgcacatgggacgctaaaactggtaaagttggtaagttgtggggcgaaattaaataa

SEQ ID NO: 68 - protein, 425 aa, Artificial Sequence
  artificial construct
MRGSHHHHHHGSGSGSGIEGRAATHEHSAQWLNNYKKGYGYGPYPLGINGGMHYGVDFFMNIGTPVKAISSGKIVEAGWSNYGGGNQIGLIENDGVHRQWYMHLSKYNVKVGDYVKAGQIIGWSGSTGYSTAPHLHFQRMVNSFSNSTAQDPMPFLKSAGYGKAGGTVTPTPNTGELAATHEHSAQWLNNYKKGYGYGPYPLGINGGMHYGVDFFMNIGTPVKAISSGKIVEAGWSNYGGGNQIGLIENDGVHRQWYMHLSKYNVKVGDYVKAGQIIGWSGSTGYSTAPHLHFQRMVNSFSNSTAQDPMPFLKSAGYGKAGGTVTPTPNTGWKQNKDGIWYKAEHASFTVTAPEGIITRYKGPWTGHPQAGVLQKGQTIKYDEVQKFDGHVWVSWETFEGETVYMPVRTWDAKTGKVGKLWGEIK

SEQ ID NO: 69 - DNA, 1272 bp, Artificial Sequence
  artificial construct
atgagaggatcgcatcaccatcaccatcacggatctggctctggatctggtatcgagggaagggctgcaacacatgaacattcagcacaatggttgaataattacaaaaaaggatatggttacggtccttatccattaggtataaatggcggtatgcactacggagttgatttttttatgaatattggaacaccagtaaaagctatttcaagcggaaaaatagttgaagctggttggagtaattacggaggaggtaatcaaataggtcttattgaaaatgatggagtgcatagacaatggtatatgcatctaagtaaatataatgttaaagtaggagattatgtcaaagctggtcaaataatcggttggtctggaagcactggttattctacagcaccacatttacacttccaaagaatggttaattcattttcaaattcaactgcccaagatccaatgcctttcttaaagagcgcaggatatggaaaagcaggtggtacagtaactccaacgccgaatacaggtgagctcgctgcaacacatgaacattcagcacaatggttgaataattacaaaaaaggatatggttacggtccttatccattaggtataaatggcggtatgcactacggagttgatttttttatgaatattggaacaccagtaaaagctatttcaagcggaaaaatagttgaagctggttggagtaattacggaggaggtaatcaaataggtcttattgaaaatgatggagtgcatagacaatggtatatgcatctaagtaaatataatgttaaagtaggagattatgtcaaagctggtcaaataatcggttggtctggaagcactggttattctacagcaccacatttacacttccaaagaatggttaattcattttcaaattcaactgcccaagatccaatgcctttcttaaagagcgcaggatatggaaaagcaggtggtacagtaactccaacgccgaatacaggttggaaaacaaacaaatatggcacactatataaatcagagtcagctagcttcacacctaatacagatataataacaagaacgactggtccatttagaagcatgccgcagtcaggagtcttaaaagcaggtcaaacaattcattatgatgaagtgatgaaacaagacggtcatgtttgggtaggttatacaggtaacagtggccaacgtatttacttgcctgtaagaacatggaataaatctactaatactttaggtgttctttggggaactataaagtaa

SEQ ID NO: 70 - protein, 423 aa, Artificial Sequence
  artificial construct
MRGSHHHHHHGSGSGSGIEGRAATHEHSAQWLNNYKKGYGYGPYPLGINGGMHYGVDFFMNIGTPVKAISSGKIVEAGWSNYGGGNQIGLIENDGVHRQWYMHLSKYNVKVGDYVKAGQIIGWSGSTGYSTAPHLHFQRMVNSFSNSTAQDPMPFLKSAGYGKAGGTVTPTPNTGELAATHEHSAQWLNNYKKGYGYGPYPLGINGGMHYGVDFFMNIGTPVKAISSGKIVEAGWSNYGGGNQIGLIENDGVHRQWYMHLSKYNVKVGDYVKAGQIIGWSGSTGYSTAPHLHFQRMVNSFSNSTAQDPMPFLKSAGYGKAGGTVTPTPNTGWKTNKYGTLYKSESASFTPNTDIITRTTGPFRSMPQSGVLKAGQTIHYDEVMKQDGHVWVGYTGNSGQRIYLPVRTWNKSTNTLGVLWGTIK

SEQ ID NO: 71 - DNA, 1278 bp, Artificial Sequence
  artificial construct
atgagaggatcgcatcaccatcaccatcacggatctggctctggatctggtatcgagggaagggctgcaacacatgaacattcagcacaatggttgaataattacaaaaaaggatatggttacggtccttatccattaggtataaatggcggtatgcactacggagttgatttttttatgaatattggaacaccagtaaaagctatttcaagcggaaaaatagttgaagctggttggagtaattacggaggaggtaatcaaataggtcttattgaaaatgatggagtgcatagacaatggtatatgcatctaagtaaatataatgttaaagtaggagattatgtcaaagctggtcaaataatcggttggtctggaagcactggttattctacagcaccacatttacacttccaaagaatggttaattcattttcaaattcaactgcccaagatccaatgcctttcttaaagagcgcaggatatggaaaagcaggtggtacagtaactccaacgccgaatacaggtgagctcgctgcaacacatgaacattcagcacaatggttgaataattacaaaaaaggatatggttacggtccttatccattaggtataaatggcggtatgcactacggagttgatttttttatgaatattggaacaccagtaaaagctatttcaagcggaaaaatagttgaagctggttggagtaattacggaggaggtaatcaaataggtcttattgaaaatgatggagtgcatagacaatggtatatgcatctaagtaaatataatgttaaagtaggagattatgtcaaagctggtcaaataatcggttggtctggaagcactggttattctacagcaccacatttacacttccaaagaatggttaattcattttcaaattcaactgcccaagatccaatgcctttcttaaagagcgcaggatatggaaaagcaggtggtacagtaactccaacgccgaatacaggtggtaaatctgcaagtaaaataacagttggaagtaaagcgccttataaccttaaatggtcaaaaggtgcttattttaatgcgaaaatcgacggcttaggtgctacttcagccactagatacggtgataatcgtactaactatagattcgatgttggacaggctgtatacgcgcctggaacattaatatatgtgtttgaaattatagatggttggtgtcgcatttattggaacaatcataatgagtggatatggcatgagagattgattgtgaaagaagtgttttaa

SEQ ID NO: 72 - protein, 425 aa, Artificial Sequence
  artificial construct
MRGSHHHHHHGSGSGSGIEGRAATHEHSAQWLNNYKKGYGYGPYPLGINGGMHYGVDFFMNIGTPVKAISSGKIVEAGWSNYGGGNQIGLIENDGVHRQWYMHLSKYNVKVGDYVKAGQIIGWSGSTGYSTAPHLHFQRMVNSFSNSTAQDPMPFLKSAGYGKAGGTVTPTPNTGELAATHEHSAQWLNNYKKGYGYGPYPLGINGGMHYGVDFFMNIGTPVKAISSGKIVEAGWSNYGGGNQIGLIENDGVHRQWYMHLSKYNVKVGDYVKAGQIIGWSGSTGYSTAPHLHFQRMVNSFSNSTAQDPMPFLKSAGYGKAGGTVTPTPNTGGKSASKITVGSKAPYNLKWSKGAYFNAKIDGLGATSATRYGDNRTNYRFDVGQAVYAPGTLIYVFEIIDGWCRIYWNNHNEWIWHERLIVKEVF

SEQ ID NO: 73 - protein, 506 aa, Artificial Sequence
  artificial construct
MAATHEHSAQWLNNYKKGYGYGPYPLGINGGMHYGVDFFMNIGTPVKAISSGKIVEAGWSNYGGGNQIGLIENDGVHRQWYMHLSKYNVKVGDYVKAGQIIGWSGSTGYSTAPHLHFQRMVNSFSNSTAQDPMPFLKSAGYGKAGGTVTPTPNTGELLRPKDAKKDEKSQVCSGLAMEKYDITNLNAKQDKSKNGSVKELKHIYSNHIKGNKITAPKPSIQGVVIHNDYGSMTPSQYLPWLYARENNGTHVNGWASVYANRNEVLWYHPTDYVEWHCGNQWANANLIGFEVCESYPGRISDKLFLENEEATLKVAADVMKSYGLPVNRNTVRLHNEFFGTSCPHRSWDLHVGKGEPYTTTNINKMKDYFIKRIKHYYDGGKLEVSKAATIKQSDVKQEVKKQEAKQIVKATDWKQNKDGIWYKAEHASFTVTAPEGIITRYKGPWTGHPQAGVLQKGQTIKYDEVQKFDGHVWVSWETFEGETVYMPVRTWDAKTGKVGKLWGEIK

SEQ ID NO: 74 - protein, 462 aa, Artificial Sequence
  artificial construct
MAATHEHSAQWLNNYKKGYGYGPYPLGINGGMHYGVDFFMNIGTPVKAISSGKIVEAGWSNYGGGNQIGLIENDGVHRQWYMHLSKYNVKVGDYVKAGQIIGWSGSTGYSTAPHLHFQRMVNSFSNSTAQDPMPFLKSAGYGKAGGTVTPTPNTGLKHIYSNHIKGNKITAPKPSIQGVVIHNDYGSMTPSQYLPWLYARENNGTHVNGWASVYANRNEVLWYHPTDYVEWHCGNQWANANLIGFEVCESYPGRISDKLFLENEEATLKVAADVMKSYGLPVNRNTVRLHNEFFGTSCPHRSWDLHVGKGEPYTTTNINKMKDYFIKRIKHYYDGGKLEVSKAATIKQSDVKQEVKKQEAKQIVKATDWKQNKDGIWYKAEHASFTVTAPEGIITRYKGPWTGHPQAGVLQKGQTIKYDEVQKFDGHVWVSWETFEGETVYMPVRTWDAKTGKVGKLWGEIK

SEQ ID NO: 75 - protein, 10 aa, Artificial Sequence
  Synthetic peptide
ELAGIGILTV